European Patent Application EP 4 545 548 A1, published April 30, 2025. Title: INSECT NEUROPEPTIDES 2. Applicant: SOLASTA Bio Limited. The sequence listing filed with the application follows.

SEQUENCE LISTING (16 sequences)

SEQ ID NO: 1 - protein, 11 aa, synthetic construct
  source 1..11: note = Z peptide
AIMARPQVPRL

SEQ ID NO: 2 - protein, 11 aa, synthetic construct
  source 1..11: note = SB-P-47
  MOD_RES 11: note = leucinamide
  MOD_RES 1: note = pyroglutamyl-alanine
AIMARPQVPRL

SEQ ID NO: 3 - protein, 12 aa, synthetic construct
  source 1..12: note = SB-P-46
  MOD_RES 12: note = leucinamide
SPPYSPPFSPRL

SEQ ID NO: 4 - protein, 8 aa, synthetic construct
  source 1..8: note = SB-P-49
  MOD_RES 8: note = leucinamide
SVPFKPRL

SEQ ID NO: 5 - protein, 19 aa, synthetic construct
  source 1..19: note = SB-P-51
  MOD_RES 19: note = leucinamide
LRQLQSNGEPAYRVRTPRL

SEQ ID NO: 6 - protein, 16 aa, synthetic construct
  source 1..16: note = SB-P-80
  MOD_RES 16: note = leucinamide
NADEDQQQSVDFTPRL

SEQ ID NO: 7 - protein, 10 aa, synthetic construct
  source 1..10: note = SB-P-81
  MOD_RES 10: note = leucinamide
GGSMTFSPRL

SEQ ID NO: 8 - protein, 8 aa, synthetic construct
  source 1..8: note = SB-P-70
  MOD_RES 8: note = glycinamide
KVKFSAWG

SEQ ID NO: 9 - protein, 10 aa, synthetic construct
  source 1..10: note = SB-P-65
  MOD_RES 10: note = glycinamide
RQKTVFSSWG

SEQ ID NO: 10 - protein, 7 aa, synthetic construct
  source 1..7: note = SB-P-66
  MOD_RES 7: note = glycinamide
PAFSSWG

SEQ ID NO: 11 - protein, 9 aa, synthetic construct
  source 1..9: note = SB-P-86
  MOD_RES 9: note = glycinamide
  MOD_RES 1: note = pyroglutamyl-leucine
LTFTSSWGG

SEQ ID NO: 12 - protein, 8 aa, synthetic construct
  source 1..8: note = SB-P-039
  MOD_RES 1: note = palmitoyl-glutamine
  MOD_RES 8: note = tryptophanamide
QLTFSPDW

SEQ ID NO: 13 - protein, 7 aa, synthetic construct
  source 1..7: note = SB-P-042
  MOD_RES 1: note = pyroglutamyl-leucine
  MOD_RES 7: note = tryptophanamide
LTFSPDW

SEQ ID NO: 14 - protein, 6 aa, synthetic construct
  source 1..6: note = SB-P-69
  MOD_RES 6: note = glycinamide
NFSPWG

SEQ ID NO: 15 - protein, 19 aa, synthetic construct
  source 1..19: note = SB-P-48
  MOD_RES 19: note = leucinamide
EQNVQSNGEPAYRVRTPRL

SEQ ID NO: 16 - protein, 8 aa, synthetic construct
  source 1..8: note = SB-P-41
  MOD_RES 8: note = tryptophanamide
QLTFSPDW